European Patent Specification EP 3 428 277 B1, published May 10, 2023. Title: Luminescent Protein. Applicant: NATIONAL INSTITUTE OF ADVANCED INDUSTRIAL SCIENCE AND TECHNOLOGY. The sequence listing filed with the application follows.

SEQUENCE LISTING (12 sequences)

SEQ ID NO: 1 - DNA, 1252 bp, Odontosyllis undecimdonta
tgagtaacagtgctaacttcatcatcacaagaagatacttctcagcttgtattgaagatgaagttagcactgttactcagcattggatgttgcctggttgccgtgaactttgctttaagggctactatcataagatgtcttaggaaaactagaagttggtcagaaatagattgtacaccacatcaggacaagctatatgaagactttgacaggatctgggcaggagattacctgtcggtatttgctgaatggttagataatcccatccctcgagagtggtctgaggaaagactggccacatactgcatagagagggaatgtcacactaatcaagctatggttgactatatgaatatacatgggtatgcccctttttgcatggaaaggagtgttgaagactgggtgaatgctagattctggactagatgtaaggttagaactgaccgtagtttagaactggcacctgaagaatatgccacctacttttgttataaggtgtttcgtgtacaggatcctaaaatagcttgtccctcgatggatgtgatcctttcacctaacaaactgactgtacaacaaatgatgcagaataaggaaataagaggagttgtagaggatagatctgagcaatggtgggttggactaatgagagaaatatcgcatctgtctaaggacttgaatggtgtgaaacaattccattatggatggatcataaacacagctacacaaaagaatgtggttcctttgtggtcacgttatcaggggcctactattccagtaagaagagacatgcctagaatcattaatgccatgtctaatggaggaggaaacatcaccttgggagatattcgaaatttccactgctcagctgatccagacagtgttgctgtcatctgccctgagtttggtttcttgtcctatagtccagctgaaactatagttatggttccagtaaatggattaatcctgatgggaatgacacaatctgcagatggagtacccttcgtaaaatctgcactatttgctgagatgtataacctacaacagtaagagatcatccaggacactgaggctgaatgtggtcattatttatacacagtttattcccttaatctttgcaacattataatttagttttgataatcatgatgattaatgtagatataatataaacatatattatatgatcagatactcttactattctttttatgctttgtttttttattaaattctccgcattttctattctgat

SEQ ID NO: 2 - protein, 329 aa, Odontosyllis undecimdonta
MKLALLLSIGCCLVAVNFALRATIIRCLRKTRSWSEIDCTPHQDKLYEDFDRIWAGDYLSVFAEWLDNPIPREWSEERLATYCIERECHTNQAMVDYMNIHGYAPFCMERSVEDWVNARFWTRCKVRTDRSLELAPEEYATYFCYKVFRVQDPKIACPSMDVILSPNKLTVQQMMQNKEIRGVVEDRSEQWWVGLMREISHLSKDLNGVKQFHYGWIINTATQKNVVPLWSRYQGPTIPVRRDMPRIINAMSNGGGNITLGDIRNFHCSPDPDSVAVICPEFGFLSYSPAETIVMVPVNGLILMGMTQSTDGVPFVKSALFAEMYNLQQ

SEQ ID NO: 3 - DNA, 27 bp, Artificial sequence
  PCR primer
catatgaagttagcactgttactcagc

SEQ ID NO: 4 - DNA, 30 bp, Artificial sequence
  PCR primer
tctagactgttgtaggttatacatctcagc

SEQ ID NO: 5 - DNA, 4805 bp, Odontosyllis undecimdonta
atgaagttagcactgttactcagcattggatgttgcctggttgccgtcaactttgctttaagggctactatcataagatgtcttagggtaagacttcagaaactcatattgaccatgagggcctctataataatatttcttaatgtaagactacagaagctcatattgaccttaagggtctctataataatatttcttaatgtaagactacagaagctcatattgaccttgagtctctataataatatttcttaatgtaagacaacagaagctcatattgaccttgagggtctctataataatacatataattacatcttgatttaattatttctcttagaaaactagaagttggtcagaaatagattgtacaccacatcaggacaagctatatgaggactttgacaggatctgggctggagattacctgtcagtatttgccgaatggttagataatcccatccctcgagagtggtctgaggaaagactggccacatactgcatagagagggaatgtcacactaatcaagctatggtggactatatgaatatacatggggtaaagttttagcacatgtttttatgtacagtatctgctttattatggttttaatcgtagtacattttatatgtatagtatctgctttattatggttttaatcttagtacatgtttatatttacagtatgccccttataatggttttaatcttggtacatgtttgtacttacagtatctgctttattatggttttaatcttagtacatgtttgtatttacagtatctgccttattatggttttaatcttagtacatgttttgtacttacagtatgcccctttttgcatggaaaggagtgttgaagactgggtgaatgctagattctggactaggtatgcagtttcatcaaatgtttatatcaataaaatataatgcttagtaaagcagctgccaatccgggttaagtattttttttccaagcacatttgtacaaaacggcatagtatccatagtgtagggacaattctttggaatggtcaattctacactgcagtcagtgattgatagttataaatatgtcagattcagcaattaatggttaatgaatgaattgctatttaccacaatgttgtaccattacaacattcagctaggctgtccagccatcaaacacatactcagtgtgctccttctacatatttgtactgatctgcactacatggaagttttttctagactagtggtgcatgtattgcatatgactgtactttagttctaggaaaggagagtgttaactacacccttgagtagttataggcaacaaacatgaagttaccttttcaattgaaccatgttgacagtgggctgtatacagctcggaagtagcctaagcagggtaaaagtagccaataaatcatattgtggcaaacagcaattccttttgcctcataaataattaatgatggatattccaaaaagtgtctaggggagagtgagagacttttttgaagaaattgtatggttttagataacagtcatactatatacaaatagttgcagccaaatctcttcctttcttcaagataatttgtttcttcatcatttactacattcccaaattgttctgtggcaagttgaaaataggaaaaacatcctacaaattggattctgattcctcataacctaaggcaaactcatctccttgattcagaatgtagcaataatctacccatattacccatgtaatttgtttcattgaccttcaaatcaaatgctctgttattcctcctcattatcaataatatgattacttttgcagatgtaaggttagaactgatcgtagtttagaactggcacctgaagaatatgccacctacttttgttataaggtgtttcgtgtacaggatcctaaaatagcttgtccctcgatggatgtgatcctttcacctaacaaactgactgtacaacaaatgatgcaaaataaggtaagaaccacccctaagccaggccatacttatttgatagttcagactcatgtgcaggaaggagtgccctgtgacatactgcatatattttgaaccaaaatatttgtatacttgtagttaaaatcaatgtgagcgagactttagataagagccaatggttcattagatagtccaaatcaatgtgagcgagactttagagaagagccaatggttcggtagatagtccaaatcaatctgagctagactttagagaagagcaatggttcattagatagttcaaatcaatatgagctagactttagagaagagccaatggttcggtagatagtccaaatcaatctgcgctagactttagagaagagcaatggttcattagatagtccaaatcaatatgtttctagactttagagaagagccaatggttcattagatagttcaaatcaatatgagctagactttagagaagagccaatggttcattagatagttcaaatcaatatgagctagactttagagaagagcaatggttcagtagatagttcaaatcaatatgagctagactttagagaagagccaatacaatatgagctagactttagagaaggccaagtggtataaggtgcaattaatctcaataaaagagtcaaacctttgagaagatagcttgaatcttaagaaggaaggcatcttaatagaagatccacaagattgtttaaattaagggagacacagctaaacgaaaaagccaagaaggctaatgaagcggtactgacatttttacttgtttataccacaggaaataagaggagttgtagaggatagatctgagcaatggtgggttggactaatgagagaaatatcgcatctgtctaaggacttgaatggtgtgaaacaattccattatggatggatcataaacacagctacacaaaagaatgtggttcctttgtggtcacgttatcagggggtaagaaattctacattataagaatgtgatttattaagcttgctcatcactttgtgttggcacattgtatttgctactgctagatccttgagtgaacttaactcatataacttagaatctgcatgcatattttcaactagacatagtaataatattttacataaatcacttccttgcataacagaaaatgttctgaattttgtattaaacagtccttaactctggaccctctaaacattaaaaatactgttggaccctaagtccattttaaagtgagctaagtcaagtcccactgttatagcaattttaaatttaaatgaagcctccagtcaagattgcaaaaagtctcagaaggatacagatttgtgatccccctctaaaatttgtaaataacaaaatgaatagatcttgacatagccatacatatttgcatatgactatccaaaggtttttggagagagataatttttctcctcccattaggaggtgtttttgaggtaaccaaaatattaccccccctccccatggatatggatgaggggtatacttttctttcatatttcaatctaaaaatccctttttccaacttaaacaatttgaacttagtttacactaagtcaactaatttagtatcccatccttttacctacttgtagtctgaaactgtgtggtattaggaagaatcacagtttaaatgtacatgagctattttagcccaatacaaactaatgatatttttttcagccctactattccagtaagaagagacatgcctagaatcattaatgccatgtctaatggaggaggaaacattaccttgggaggtaaataaataaataaaaacttgtataaacataaatattgcatcactgaagcaaataaacctatctacctgctgaagctgctaaactggatattcactgaacatttgtaatatttggtttattattatgttgatgggattcaaataataataaaatttacaaatatatgttctgtaaaattggcagccagccaggaaaaacgataaaatatagatgtatattgtattgttgtcactttttatccaatttagagaccaggatgaaacatttagtcaataataaacatatatatatagttattttattaaatctcaagctacaattataagtgctggtaaatagttgatcaataaccatttttcatgaaataaataaaataaaatgatcagtaaaatctcaatacatcatcataactacagataaattattttgtagatattcgaaatttccactgctctcctgatccagacagtgttgctgtcatctgccctgagttcggtttcttgtcctatagcccagctgaaactatagtaatggttccagtaaatggatgtaagattgcatttccttattatctaaataataattatgtagagtactacttcccccttcaagctgtttatccagtctttgttatctcatattcaatattctgtgtaataagtttaaccctcaagaatagaaatgtaagcctgcaggtgtagtaatgacctcctgtaggtgtagtaatggcctcctgtaaccagtagtattaatcgtataaagtatactattgtcattacaacacatctagaactgtggaggccaaaagtggaaattgtaaaaccatccacaataaactggtgctatataaaaacgtagagtaagggatgtacaattcttaaagtatcaaacaatgacaccaacacaccatcactattgccataactatatttctatttcagtaatcctgatgggaatgacacaatctacagatggagtacctttcgtaaaatctgccctatttgctgagatgtataacctacaacag

SEQ ID NO: 6 - DNA, 29 bp, Artificial sequence
  PCR primer
acaagcttatgaagttagcactgttactc

SEQ ID NO: 7 - DNA, 29 bp, Artificial sequence
  PCR primer
aacccgggttactgttgtaggttatacat

SEQ ID NO: 8 - DNA, 21 bp, Artificial sequence
  PCR primer
atgaagttagcactgttactc

SEQ ID NO: 9 - DNA, 21 bp, Artificial sequence
  PCR primer
ggtagatcaattctgacggtt

SEQ ID NO: 10 - DNA, 987 bp, Odontosyllis undecimdonta
atgaagttagcactgttactcagcattggatgttgcctggttgccgtcaactttgctttaagggctactatcataagatgtcttaggaaaactagaagttggtcagaaatagattgtacaccacatcaggacaagctatatgaggactttgacaggatctgggctggagattacctgtcagtatttgccgaatggttagataatcccatccctcgagagtggtctgaggaaagactggccacatactgcatagagagggaatgtcacactaatcaagctatggtggactatatgaatatacatgggtatgcccctttttgcatggaaaggagtgttgaagactgggtgaatgctagattctggactaggtgtaaggttagaactgatcgtagtttagaactggcacctgaagaatatgccacctacttttgttataaggtgtttcgtgtacaggatcctaaaatagcttgtccctcgatggatgtgatcctttcacctaacaaactgactgtacaacaaatgatgcaaaataaggaaataagaggagttgtagaggatagatctgagcaatggtgggttggactaatgagagaaatatcgcatctgtctaaggacttgaatggtgtgaaacaattccattatggatggatcataaacacagctacacaaaagaatgtggttcctttgtggtcacgttatcaggggcctactattccagtaagaagagacatgcctagaatcattaatgccatgtctaatggaggaggaaacattaccttgggagatattcgaaatttccactgctctcctgatccagacagtgttgctgtcatctgccctgagttcggtttcttgtcctatagcccagctgaaactatagtaatggttccagtaaatggattaatcctgatgggaatgacacaatctacagatggagtacctttcgtaaaatctgccctatttgctgagatgtataacctacaacag

SEQ ID NO: 11 - protein, 8 aa, Artificial sequence
  MS-MS result
WEDWVNAR

SEQ ID NO: 12 - protein, 8 aa, Artificial sequence
  MS/MS result
WEDWVNAR